European Patent Application EP 4 316 245 A1, published February 7, 2024. Title: GENE EXPRESSION ENHANCER AND PHOTOSYNTHESIS ACTIVATOR. Applicant: Denka Company Limited Tohoku University. The sequence listing filed with the application follows.

SEQUENCE LISTING (6 sequences)

SEQ ID NO: 1 - DNA, 21 bp, Artificial Sequence
  ACT2 primer
cattgtgctcagtggtggttc

SEQ ID NO: 2 - DNA, 21 bp, Artificial Sequence
  ACT2 primer
tctgctggaaggtgctaagtg

SEQ ID NO: 3 - DNA, 20 bp, Artificial Sequence
  DnaJ primer
ctacgatccaggagatcaag

SEQ ID NO: 4 - DNA, 20 bp, Artificial Sequence
  DnaJ primer
gacgtgtccttctgatcaat

SEQ ID NO: 5 - DNA, 20 bp, Artificial Sequence
  NR primer
cgtaggccgtactttcaagc

SEQ ID NO: 6 - DNA, 20 bp, Artificial Sequence
  NR primer
catcgtcatcctcgtcttca